European Patent Specification EP 3 568 415 B1, published January 22, 2025. Title: ANTIBODIES TO T CELL IMMUNORECEPTOR WITH IG AND ITIM DOMAINS (TIGIT) AND USES THEREOF. Applicant: I-Mab. The sequence listing filed with the application follows.

SEQUENCE LISTING (80 sequences)

SEQ ID NO: 1 - protein, 119 aa, Artificial Sequence
  Synthetic
EVQLQQSGPELVKPGASVKISCKTSGYTFTENTMHWVKQSHGKSLEWIGGINPNQGGNRNNQKFKGKATLTVDKSSSTAYMELRSLTSEDSAVYYCARSGLRDYAMDYWGQGTSVTVSS

SEQ ID NO: 2 - protein, 107 aa, Artificial Sequence
  Synthetic
DIVMTQSHKFMSTSVGDRVSITCKASQHVSTAVVWYQQKPGQSPKLLIYSPSYRYTGVPDRFTGSGSGTDFTFTISSVQAEDLAVYYCQQHYSTPWTFGGGTKLEIK

SEQ ID NO: 3 - protein, 118 aa, Artificial Sequence
  Synthetic
DVQLQESGPGLVKPSQSLSLTCTVTGYSITSDYAWNWIRQFPGNKLEWMGYISYSGNTRYNPSLKSRISITRDTSKNQFFLQFNSVTTEDTATYYCSRKYYGSWFPYWGQGTLVTVSA

SEQ ID NO: 4 - protein, 107 aa, Artificial Sequence
  Synthetic
DIVMTQSHKFMSTSVGDRVSITCKASQDVFTAVAWYQQKPGQSPKLLIYSASYRYTGVPDRFTGSGSGTDFTFTISSVQAEDLAVYYCQQHYSTPWTFGGGTRLEIK

SEQ ID NO: 5 - protein, 119 aa, Artificial Sequence
  Synthetic
EFQLQQSGPELVKPGASVKISCRASGYSFTAYSMNWVQQTNGKSLEWIGVINPKFGTINYNQKFKGKATLTVDQSSSAAYIQLNSLTSEDSAVYFCARNGNFAWYFDVWGTGTTVTVSS

SEQ ID NO: 6 - protein, 107 aa, Artificial Sequence
  Synthetic
DIQMTQSPASLSASVGETVTITCRASENIFSYLAWYQQKQGKSPQLLVYNAKTLPEGVPSRFSGSGSGTQFSLKINSLQSEDFGSYYCQHHYGVPWTFGGGTKLEIK

SEQ ID NO: 7 - protein, 119 aa, Artificial Sequence
  Synthetic
EFQLQQSGPELVKPGASVKISCRASGYSFTAYSINWVQQTNGKSLEWIGVINPKFGTINYNQKFKGKATLTVDQSSSAAYMQLNSLTSEDSAVYFCARNGNFAWYFDVWGTGTTVTVSS

SEQ ID NO: 8 - protein, 107 aa, Artificial Sequence
  Synthetic
DIQMTQSPASLSASVGETVTITCRAGENIYSYLAWYQQKQGKSPQLLVYNAKTLPEGVPSRFSGSGSGTQFSLKINSLQSEDFGSYYCQHHYGVPWTFGGGTKLEIK

SEQ ID NO: 9 - protein, 119 aa, Artificial Sequence
  Synthetic
EFQLQQSGPELVKPGASVKISCRASGYSFTAYSMNWVQQTNGKSLEWIGVINPKFGTTNYNQKFRDKATLTVDHSSSAAYMQLNSLTSEDSAVYFCARNGNFAWYFDVWGTGTTVTVSS

SEQ ID NO: 10 - protein, 107 aa, Artificial Sequence
  Synthetic
DIQMTQSPASLSASVGETVTITCRASENIFSYLAWYQQKQGKSPQLLAYNAETLAEGVPSRFSGSGSGTQFSLKISSLQSEDFGSYYCQHHFGVPWTFGGGTNLEIK

SEQ ID NO: 11 - protein, 119 aa, Artificial Sequence
  Synthetic
EVQLVESGGGLVMPGGSLKLSCAASGFTFSGFVMSWVRQTPEKRLEWVATINDAGTYTYYSDNLKGRFTISRDNAKNNLYLQMSHLKSEDAGMYYCARDGGLRAWFPYWGPGTLVTVSA

SEQ ID NO: 12 - protein, 107 aa, Artificial Sequence
  Synthetic
DIQLTQSPASLSASVGETVTITCRASENIYSYLAWYQLKQGKSPQLLVFNTKTLAEGVPSRFSGSGSGTQFSLRIDSLQLEDFGSFYCQHHIGSPRTFGGGTTLEIR

SEQ ID NO: 13 - protein, 119 aa, Artificial Sequence
  Synthetic
EFQLQQSGPELVKPGASVKISCRASGYSFTAYSMNWVQQTNGKSLEWIGVINPKFGTINYNQKFKDKATLTVDHSSSAAYMQLNSLTSEDSAVYFCARNGNFAWYFDVWGTGTTVTVSS

SEQ ID NO: 14 - protein, 107 aa, Artificial Sequence
  Synthetic
DIQMTQSPASLSASVGETVTITCRASESIFSYLAWYQQKQGKSPQLLAYNAETLAEGVPSRFSGSGSGTQFSLKINSLQSEDFGIYYCQHHFGVPWTFGGGTKLEIK

SEQ ID NO: 15 - protein, 119 aa, Artificial Sequence
  Synthetic
EIQLQQTGPELVKPGASVNISCKASGYSFTDYIMIWVKQSHGKSLEWIGNIHPYFGNSHYNLKFKGKATLTVDKSSTTAYMQLNSLTSEDSAVYYCARRGITSAHFDYWGQGTTLTVSS

SEQ ID NO: 16 - protein, 111 aa, Artificial Sequence
  Synthetic
DIVLTQSPASLAVSLGQRATISCRASKSVSTSGYSYMHWYQQKPGQPPKLLIYRASNLESGVPARFSGSGSGTDFTLNIHPVEEEDAATYYCQHSGDLPWTFGGGTKLEIK

SEQ ID NO: 17 - protein, 115 aa, Artificial Sequence
  Synthetic
EVQLQQSGPELVKPGASVKISCKTSGYTFSDYTLHWVKQSHGKNLEWIGGFNPNNGGTNYNQKFKVKASLTIDKSSNTVYMELRSLSSEDSAVYYCARNWAFDYWGQGTTLTVSS

SEQ ID NO: 18 - protein, 107 aa, Artificial Sequence
  Synthetic
DIVMTQSHKIMSTSLGDRVNITCKASQHVSTAVAWYQQRPGQSPRLLIYSASYRHTGVPDRFTGSGSGTDITFTISSVQTEDLAVYYCQQYYTTPWTFGGGTKLEIK

SEQ ID NO: 19 - protein, 115 aa, Artificial Sequence
  Synthetic
QIQLVQSGPELKKPGETVKISCKASGYTFTAYGMSWVKQTPGKGLKWMGWINTYSGVPTYADDFKGRFAFSLETSASTAYLQINNLKNEDTATYFCTRGDTGGYWGQGATLTVSS

SEQ ID NO: 20 - protein, 105 aa, Artificial Sequence
  Synthetic
QIVLTQSPAIMSASLGEEITLTCSARSSVSDMHWYQQKSGTSPKLLIYSTSNLASGVPSRFSGSGSGTFFSLTISSVEAEDAADYYCHQWGGYPTFGGGTKLEIK

SEQ ID NO: 21 - protein, 119 aa, Artificial Sequence
  Synthetic
QIQLVQSGPELKKPGETVKISCKASGYTFTAYGMGWVKQAPGKGLKWMGWINTYSGVPTYADDFKGRFAFSLESSASTAYLQINNLKNEDTATYFCARGIYFGNYFDYWGQGTTLTVSS

SEQ ID NO: 22 - protein, 107 aa, Artificial Sequence
  Synthetic
DIQMTQSPASLSASVGETVTITCRASEIIYTFLAWYQQKQGKSPQLLVYNANTLAEGVPSRFSGSGSGTQFSLKINSLQPEDFGSYYCQHHYGSPYTFGGGTTLEIK

SEQ ID NO: 23 - protein, 119 aa, Artificial Sequence
  Synthetic
QIQLIQSGPEVKKPGETVKISCKASGYTFTTYAMTWVKQAAGKGLKWMGWIHTYSGVPTYVDDFKGRFAFSLDTSANTAYLQINNLKNEDTATYFCARYDGPLYAMDFWGQGTSVTVSS

SEQ ID NO: 24 - protein, 106 aa, Artificial Sequence
  Synthetic
QIVLTQSPAIMSASPGEKVTISCSASSSVSYMFWYQQKPGSSPKSWIYRTSNLASGVPGRFSGSGSGTSYSLTISSMEAEDAATYYCQQYHSYFPTFGGGTKLEIK

SEQ ID NO: 25 - protein, 117 aa, Artificial Sequence
  Synthetic
DVQLQESGPGMVKPSQSLSLTCTVTGYSITSGYDWHWIRHFPGNKLEWMGFISDSGSTKYNPSLKSRISITHDTSKNHFFLKLNSVTSEDTATYYCARGSYWYFDVWGTGTTVTVSS

SEQ ID NO: 26 - protein, 107 aa, Artificial Sequence
  Synthetic
DIQMTQSPASLSASVGETVTITCRASENIYSYLAWYQQKQGKSPQLLVNNAKTLAEGVSSRFSGSGSGTQFSLKINSLQPEDFGSYYCQHHYGNPLMFGAGTKLELK

SEQ ID NO: 27 - protein, 119 aa, Artificial Sequence
  Synthetic
EVKLVESGGALVQPGGSLKLSCAASGFTFSDYYMYWVRQTPEKRLEWVASITKGGGSTYYPDTLKGRFTISRDNAKNTLYLQMSRLKSEDTDMYYCARQSSYDFVMDYWGQGTSVTVSS

SEQ ID NO: 28 - protein, 107 aa, Artificial Sequence
  Synthetic
DIVMTQSHKFMSTSVGDRVTITCKASQDVDTAVAWYQQKPGQSPKLLIYWASARHTGVPDRFTGSGSGTDFTLTISNVQSEDLADYFCQQYSNYPLTFGVGTKLELK

SEQ ID NO: 29 - protein, 5 aa, Artificial Sequence
  Synthetic
ENTMH

SEQ ID NO: 30 - protein, 17 aa, Artificial Sequence
  Synthetic
GINPNQGGNRNNQKFKG

SEQ ID NO: 31 - protein, 10 aa, Artificial Sequence
  Synthetic
SGLRDYAMDY

SEQ ID NO: 32 - protein, 11 aa, Artificial Sequence
  Synthetic
KASQHVSTAVV

SEQ ID NO: 33 - protein, 7 aa, Artificial Sequence
  Synthetic
SPSYRYT

SEQ ID NO: 34 - protein, 9 aa, Artificial Sequence
  Synthetic
QQHYSTPWT

SEQ ID NO: 35 - protein, 119 aa, Artificial Sequence
  Synthetic
QVQLVQSGAEVKKPGASVKVSCKASGYTFTENTMHWVRQAPGQRLEWMGGINPNQGGNRNNQKFKGRVTITRDTSASTAYMELSSLRSEDTAVYYCARSGLRDYAMDYWGQGTLVTVSS

SEQ ID NO: 36 - protein, 119 aa, Artificial Sequence
  Synthetic
QVQLVQSGAEVVKPGASVKVSCKTSGYTFTENTMHWVRQAPGQRLEWMGGINPQNGGNRNNQKFKGRVTITVDTSASTAYMELSSLRSEDTAVYYCARSGLRDYAMDYWGQGTLVTVSS

SEQ ID NO: 37 - protein, 119 aa, Artificial Sequence
  Synthetic
QVQLVQSGAEVVKPGASVKVSCKTSGYTFTENTMHWVKQAPGQRLEWIGGINPNQGGNRNNQKFKGRVTITVDTSASTAYMELSSLRSEDSAVYYCARSGLRDYAMDYWGQGTLVTVSS

SEQ ID NO: 38 - protein, 119 aa, Artificial Sequence
  Synthetic
QVQLVQSGAEVVKPGASVKISCKTSGYTFTENTMHWVKQAPGQRLEWIGGINPNQGGNRNNQKFKGRATLTVDTSASTAYMELSSLRSEDSAVYYCARSGLRDYAMDYWGQGTLVTVSS

SEQ ID NO: 39 - protein, 107 aa, Artificial Sequence
  Synthetic
DIQMTQSPSSLSASVGDRVTITCKASQHVSTAVVWYQQKPGKAPKLLIYSPSYRYTGVPSRFSGSGSGTDFTLTISSLQPEDFATYYCQQHYSTPWTFGQGTKVEIK

SEQ ID NO: 40 - protein, 107 aa, Artificial Sequence
  Synthetic
DIQMTQSPSSLSTSVGDRVTITCKASQHVSTAVVWYQQKPGKAPKLLIYSPSYRYTGVPSRFSGSGSGTDFTFTISSLQPEDFATYYCQQHYSTPWTFGQGTKVEIK

SEQ ID NO: 41 - protein, 107 aa, Artificial Sequence
  Synthetic
DIQMTQSPSSLSTSVGDRVTITCKASQHVSTAVVWYQQKPGKAPKLLIYSPSYRYTGVPSRFSGSGSGTDFTFTISSVQPEDFATYYCQQHYSTPWTFGQGTKVEIK

SEQ ID NO: 42 - protein, 107 aa, Artificial Sequence
  Synthetic
DIQMTQSPSSLSTSVGDRVTITCKASQHVSTAVVWYQQKPGKAPKLLIYSPSYRYTGVPSRFSGSGSGTDFTFTISSVQPEDFATYYCQQHYSTPWTFGQGTKLEIK

SEQ ID NO: 43 - protein, 5 aa, Artificial Sequence
  Synthetic
DYYMY

SEQ ID NO: 44 - protein, 17 aa, Artificial Sequence
  Synthetic
SITKGGGSTYYPDTLKG

SEQ ID NO: 45 - protein, 10 aa, Artificial Sequence
  Synthetic
QSSYDFVMDY

SEQ ID NO: 46 - protein, 11 aa, Artificial Sequence
  Synthetic
KASQDVDTAVA

SEQ ID NO: 47 - protein, 7 aa, Artificial Sequence
  Synthetic
WASARHT

SEQ ID NO: 48 - protein, 9 aa, Artificial Sequence
  Synthetic
QQYSNYPLT

SEQ ID NO: 49 - protein, 119 aa, Artificial Sequence
  Synthetic
EVQLVESGGGLVQPGGSLRLSCAASGFTFSDYYMYWVRQAPGKGLEWVASITKGGGSTYYPDTLKGRFTISRDNAKNSLYLQMNSLRAEDTAVYYCARQSSYDFVMDYWGQGTTVTVSS

SEQ ID NO: 50 - protein, 119 aa, Artificial Sequence
  Synthetic
EVKLVESGGGLVQPGGSLRLSCAASGFTFSDYYMYWVRQAPGKGLEWVASITKGGGSTYYPDTLKGRFTISRDNAKNSLYLQMNRLRAEDTAVYYCARQSSYDFVMDYWGQGTTVTVSS

SEQ ID NO: 51 - protein, 119 aa, Artificial Sequence
  Synthetic
EVQLVESGGGLVQPGGSLRLSCAASGFTFSDYYMYWVRQAPGKRLEWVASITKGGGSTYYPDTLKGRFTISRDNAKNSLYLQMNSLRAEDTAVYYCARQSSYDFVMDYWGQGTTVTVSS

SEQ ID NO: 52 - protein, 119 aa, Artificial Sequence
  Synthetic
EVKLVESGGGLVQPGGSLRLSCAASGFTFSDYYMYWVRQAPGKRLEWVASITKGGGSTYYPDTLKGRFTISRDNAKNSLYLQMNRLRAEDTAVYYCARQSSYDFVMDYWGQGTTVTVSS

SEQ ID NO: 53 - protein, 107 aa, Artificial Sequence
  Synthetic
DIQMTQSPSSLSASVGDRVTITCKASQDVDTAVAWYQQKPGKAPKLLIYWASARHTGVPSRFSGSGSGTDFTFTISSLQPEDIATYYCQQYSNYPLTFGQGTKLEIK

SEQ ID NO: 54 - protein, 107 aa, Artificial Sequence
  Synthetic
DIVMTQSPSSLSASVGDRVTITCKASQDVDTAVAWYQQKPGKAPKLLIYWASARHTGVPSRFSGSGSGTDFTFTISSLQPEDIATYYCQQYSNYPLTFGQGTKLEIK

SEQ ID NO: 55 - protein, 107 aa, Artificial Sequence
  Synthetic
DIQMTQSPSSLSASVGDRVTITCKASQDVDTAVAWYQQKPGQSPKLLIYWASARHTGVPSRFSGSGSGTDFTFTISSLQPEDIATYFCQQYSNYPLTFGQGTKLEIK

SEQ ID NO: 56 - protein, 107 aa, Artificial Sequence
  Synthetic
DIVMTQSPSSLSASVGDRVTITCKASQDVDTAVAWYQQKPGQSPKLLIYWASARHTGVPSRFSGSGSGTDFTFTISSLQPEDIATYFCQQYSNYPLTFGQGTKLEIK

SEQ ID NO: 57 - protein, 6 aa, Artificial Sequence
  Synthetic
SDYAWN

SEQ ID NO: 58 - protein, 16 aa, Artificial Sequence
  Synthetic
YISYSGNTRYNPSLKS

SEQ ID NO: 59 - protein, 9 aa, Artificial Sequence
  Synthetic
KYYGSWFPY

SEQ ID NO: 60 - protein, 11 aa, Artificial Sequence
  Synthetic
KASQDVFTAVA

SEQ ID NO: 61 - protein, 7 aa, Artificial Sequence
  Synthetic
SASYRYT

SEQ ID NO: 62 - protein, 9 aa, Artificial Sequence
  Synthetic
QQHYSTPWT

SEQ ID NO: 63 - protein, 118 aa, Artificial Sequence
  Synthetic
QVQLQESGPGLVKPSQTLSLTCTVSGYSITSDYAWNWIRQPPGKGLEWIGYISYSGNTRYNPSLKSRVTISVDTSKNQFSLKLSSVTAADTAVYYCARKYYGSWFPYWGQGTLVTVSS

SEQ ID NO: 64 - protein, 118 aa, Artificial Sequence
  Synthetic
QVQLQESGPGLVKPSQTLSLTCTVSGYSITSDYAWNWIRQPPGKGLEWMGYISYSGNTRYNPSLKSRVTISRDTSKNQFSLKLSSVTAADTAVYYCARKYYGSWFPYWGQGTLVTVSS

SEQ ID NO: 65 - protein, 118 aa, Artificial Sequence
  Synthetic
QVQLQESGPGLVKPSQTLSLTCTVSGYSITSDYAWNWIRQPPGKGLEWIGYISYSGNTRYNPSLKSRVTISRDTSKNQFSLKFSSVTAADTAVYYCSRKYYGSWFPYWGQGTLVTVSS

SEQ ID NO: 66 - protein, 118 aa, Artificial Sequence
  Synthetic
QVQLQESGPGLVKPSQTLSLTCTVSGYSITSDYAWNWIRQPPGKGLEWMGYISYSGNTRYNPSLKSRITISRDTSKNQFSLKFSSVTAADTAVYYCSRKYYGSWFPYWGQGTLVTVSS

SEQ ID NO: 67 - protein, 107 aa, Artificial Sequence
  Synthetic
DIQMTQSPSSLSASVGDRVTITCKASQDVFTAVAWYQQKPGKAPKLLIYSASYRYTGVPSRFSGSGSGTDFTLTISSLQPEDFATYYCQQHYSTPWTFGQGTRLEIK

SEQ ID NO: 68 - protein, 107 aa, Artificial Sequence
  Synthetic
DIQMTQSPSSLSASVGDRVTITCKASQDVFTAVAWYQQKPGKAPKLLIYSASYRYTGVPSRFSGSGSGTDFTFTISSLQPEDFATYYCQQHYSTPWTFGQGTRLEIK

SEQ ID NO: 69 - protein, 107 aa, Artificial Sequence
  Synthetic
DIQMTQSPSSLSTSVGDRVTITCKASQDVFTAVAWYQQKPGKAPKLLIYSASYRYTGVPSRFSGSGSGTDFTFTISSLQPEDFATYYCQQHYSTPWTFGQGTRLEIK

SEQ ID NO: 70 - protein, 107 aa, Artificial Sequence
  Synthetic
DIQMTQSPSSLSTSVGDRVTITCKASQDVFTAVAWYQQKPGKAPKLLIYSASYRYTGVPSRFSGSGSGTDFTFTISSVQPEDFATYYCQQHYSTPWTFGQGTRLEIK

SEQ ID NO: 71 - protein, 118 aa, Artificial Sequence
  Synthetic
QVQLQESGPGLVKPSQTLSLTCTVSGYSITDDYAWNWIRQPPGKGLEWMGYISYSGHTKYNPSLKSRVTISRDTSKNQFSLKLSSVTAADTAVYYCARKYYGGWFPRWGQGTLVTVSS

SEQ ID NO: 72 - protein, 118 aa, Artificial Sequence
  Synthetic
QVQLQESGPGLVKPSQTLSLTCTVSGYSITDDYAWNWIRQPPGKGLEWMGYISYSGNTMYNPSLKSRVTISRDTSKNQFSLKLSSVTAADTAVYYCARKYYGGWFPIWGQGTLVTVSS

SEQ ID NO: 73 - protein, 118 aa, Artificial Sequence
  Synthetic
QVQLQESGPGLVKPSQTLSLTCTVSGYSITDDYAWNWIRQPPGKGLEWMGYISYSGDTKYNPSLKSRVTISRDTSKNQFSLKLSSVTAADTAVYYCARKYYGGWFPVWGQGTLVTVSS

SEQ ID NO: 74 - protein, 118 aa, Artificial Sequence
  Synthetic
QVQLQESGPGLVKPSQTLSLTCTVSGYSITDDYAWNWIRQPPGKGLEWMGYISYSGHTRYNPSLKSRVTISRDTSKNQFSLKLSSVTAADTAVYYCARKYYGSWFPDWGQGTLVTVSS

SEQ ID NO: 75 - protein, 118 aa, Artificial Sequence
  Synthetic
QVQLQESGPGLVKPSQTLSLTCTVSGYSITDDYAWNWIRQPPGKGLEWMGYISYSGITRYNPSLKSRVTISRDTSKNQFSLKLSSVTAADTAVYYCARKYYGGWFPQWGQGTLVTVSS

SEQ ID NO: 76 - protein, 107 aa, Artificial Sequence
  Synthetic
DIQMTQSPSSLSASVGDRVTITCKASQDVFTAVAWYQQKPGKAPKLLIYSASYRPTGVPSRFSGSGSGTDFTFTISSLQPEDFATYYCQQSYSTPWTFGQGTRLEIK

SEQ ID NO: 77 - protein, 107 aa, Artificial Sequence
  Synthetic
DIQMTQSPSSLSASVGDRVTITCKASQDVFTAVAWYQQKPGKAPKLLIYSASYRHTGVPSRFSGSGSGTDFTFTISSLQPEDFATYYCQQSYSTPWTFGQGTRLEIK

SEQ ID NO: 78 - protein, 107 aa, Artificial Sequence
  Synthetic
DIQMTQSPSSLSASVGDRVTITCKASQDVFTAVAWYQQKPGKAPKLLIYSASNRNTGVPSRFSGSGSGTDFTFTISSLQPEDFATYYCQQQYSTPWTFGQGTRLEIK

SEQ ID NO: 79 - protein, 107 aa, Artificial Sequence
  Synthetic
DIQMTQSPSSLSASVGDRVTITCKASQDVFTAVAWYQQKPGKAPKLLIYSASYRMTGVPSRFSGSGSGTDFTFTISSLQPEDFATYYCQQSYSTPWTFGQGTRLEIK

SEQ ID NO: 80 - protein, 107 aa, Artificial Sequence
  Synthetic
DIQMTQSPSSLSASVGDRVTITCKASQDVFTAVAWYQQKPGKAPKLLIYSASYRDTGVPSRFSGSGSGTDFTFTISSLQPEDFATYYCQQSYSTPWTFGQGTRLEIK